European Patent Application EP 4 779 023 A1, published July 22, 2026. Title: AAV mutant having infectiveness to inner ear. Applicant: 学校法人順天堂. The sequence listing filed with the application follows.

SEQUENCE LISTING (14 sequences)

SEQ ID NO: 1 - protein, 7 aa, synthetic construct
DKAWLVG

SEQ ID NO: 2 - protein, 7 aa, synthetic construct
DGLQRRE

SEQ ID NO: 3 - protein, 7 aa, synthetic construct
GPTPRQG

SEQ ID NO: 4 - protein, 7 aa, synthetic construct
GGVAKPP

SEQ ID NO: 5 - protein, 7 aa, synthetic construct
GTYPGAG

SEQ ID NO: 6 - protein, 7 aa, synthetic construct
AYAQQAP

SEQ ID NO: 7 - protein, 7 aa, synthetic construct
NEVARRE

SEQ ID NO: 8 - DNA, 56 bp, synthetic construct
  source 1..56: mol_type = other DNA
cagtcggccagagaggcnnknnknnknnknnknnknnkgcccaggcggctgacgag

SEQ ID NO: 9 - DNA, 16 bp, synthetic construct
  source 1..16: mol_type = other DNA
ctcgtcagccgcctgg

SEQ ID NO: 10 - DNA, 25 bp, synthetic construct
  source 1..25: mol_type = other DNA
ctctctggtgaatccgggcccggcc

SEQ ID NO: 11 - DNA, 25 bp, synthetic construct
  source 1..25: mol_type = other DNA
aatctttgcccagatgggcccctga

SEQ ID NO: 12 - protein, 735 aa, Adeno-associated virus type 2 [sequence omitted]

SEQ ID NO: 13 - protein, 735 aa, synthetic construct
MAADGYLPDWLEDTLSEGIRQWWKLKPGPPPPKPAERHKDDSRGLVLPGYKYLGPFNGLDKGEPVNEADAAALEHDKAYDRQLDSGDNPYLKYNHADAEFQERLKEDTSFGGNLGRAVFQAKKRVLEPLGLVEEPVKTAPGKKRPVEHSPVEPDSSSGTGKAGQQPARKRLNFGQTGDADSVPDPQPLGQPPAAPSGLGTNTMATGSGAPMADNNEGADGVGNSSGNWHCDSTWMGDRVITTSTRTWALPTYNNHLYKQISSQSGASNDNHYFGYSTPWGYFDFNRFHCHFSPRDWQRLINNNWGFRPKRLNFKLFNIQVKEVTQNDGTTTIANNLTSTVQVFTDSEYQLPYVLGSAHQGCLPPFPADVFMVPQYGYLTLNNGSQAVGRSSFYCLEYFPSQMLRTGNNFTFSYTFEDVPFHSSYAHSQSLDRLMNPLIDQYLYYLSRTNTPSGTTTQSRLQFSQAGASDIRDQSRNWLPGPCYRQQRVSKTSADNNNSEYSWTGATKYHLNGRDSLVNPGPAMASHKDDEEKFFPQSGVLIFGKQGSEKTNVDIEKVMITDEEEIRTTNPVATEQYGSVSTNLQRGQRQAATADVNTQGVLPGMVWQDRDVYLQGPIWAKIPHTDGHFHPSPLMGGFGLKHPPPQILIKNTPVPANPSTTFSAAKFASFITQYSTGQVSVEIEWELQKENSKRWNPEIQYTSNYNKSVNVDFTVDTNGVYSEPRPIGTRYLTRNL

SEQ ID NO: 14 - protein, 744 aa, synthetic construct
MAADGYLPDWLEDTLSEGIRQWWKLKPGPPPPKPAERHKDDSRGLVLPGYKYLGPFNGLDKGEPVNEADAAALEHDKAYDRQLDSGDNPYLKYNHADAEFQERLKEDTSFGGNLGRAVFQAKKRVLEPLGLVEEPVKTAPGKKRPVEHSPVEPDSSSGTGKAGQQPARKRLNFGQTGDADSVPDPQPLGQPPAAPSGLGTNTMATGSGAPMADNNEGADGVGNSSGNWHCDSTWMGDRVITTSTRTWALPTYNNHLYKQISSQSGASNDNHYFGYSTPWGYFDFNRFHCHFSPRDWQRLINNNWGFRPKRLNFKLFNIQVKEVTQNDGTTTIANNLTSTVQVFTDSEYQLPYVLGSAHQGCLPPFPADVFMVPQYGYLTLNNGSQAVGRSSFYCLEYFPSQMLRTGNNFTFSYTFEDVPFHSSYAHSQSLDRLMNPLIDQYLYYLSRTNTPSGTTTQSRLQFSQAGASDIRDQSRNWLPGPCYRQQRVSKTSADNNNSEYSWTGATKYHLNGRDSLVNPGPAMASHKDDEEKFFPQSGVLIFGKQGSEKTNVDIEKVMITDEEEIRTTNPVATEQYGSVSTNLQRGQRGDKAWLVGAQAATADVNTQGVLPGMVWQDRDVYLQGPIWAKIPHTDGHFHPSPLMGGFGLKHPPPQILIKNTPVPANPSTTFSAAKFASFITQYSTGQVSVEIEWELQKENSKRWNPEIQYTSNYNKSVNVDFTVDTNGVYSEPRPIGTRYLTRNL